European Patent Specification EP 3 334 725 B1, published April 23, 2025. Title: MECHANISM OF RESISTANCE TO BET BROMODOMAIN INHIBITORS. Applicant: Dana-Farber Cancer Institute, Inc. Application Not Yet Assigned. The sequence listing filed with the application follows.

SEQUENCE LISTING (23 sequences)

SEQ ID NO: 1 - RNA, 25 nt, Artificial Sequence
  Synthetic Polynucleotide
  misc_feature (1)..(23): modified with r
ggaccaaauggcagccugauuacca

SEQ ID NO: 2 - RNA, 25 nt, Artificial Sequence
  Synthetic Polynucleotide
  misc_feature (1)..(23): modified with r
gcaccagcuggcuguggguccugag

SEQ ID NO: 3 - RNA, 25 nt, Artificial Sequence
  Synthetic Polynucleotide
  misc_feature (1)..(23): modified with r
cuggcacugacuuugccuugaacag

SEQ ID NO: 4 - DNA, 25 bp, Artificial Sequence
  Synthetic Polynucleotide
  misc_feature (1)..(23): modified with r
ccuccagacacaauggcacugcuta

SEQ ID NO: 5 - RNA, 18 nt, Artificial Sequence
  Synthetic Polynucleotide
  misc_feature (1)..(18): modified with r
cagaugacauagugcuaa

SEQ ID NO: 6 - RNA, 18 nt, Artificial Sequence
  Synthetic Polynucleotide
  misc_feature (1)..(18): modified with r
gcuuugucaacacgcauu

SEQ ID NO: 7 - RNA, 18 nt, Artificial Sequence
  Synthetic Polynucleotide
  misc_feature (1)..(18): modified with r
ccauguucaccaacuguu

SEQ ID NO: 8 - RNA, 18 nt, Artificial Sequence
  Synthetic Polynucleotide
  misc_feature (1)..(18): modified with r
gcaauggcacgaaagcua

SEQ ID NO: 9 - RNA, 18 nt, Artificial Sequence
  Synthetic Polynucleotide
  misc_feature (1)..(18): modified with r
gcucaagacacuauggaa

SEQ ID NO: 10 - RNA, 18 nt, Artificial Sequence
  Synthetic Polynucleotide
  misc_feature (1)..(18): modified with r
ugaucacaaucaagucua

SEQ ID NO: 11 - DNA, 52 bp, Artificial Sequence
  Synthetic Polynucleotide
ctatgtttacaaattgttacatctacgccaagcctggagatgacatagtctt

SEQ ID NO: 12 - DNA, 40 bp, Artificial Sequence
  Synthetic Polynucleotide
gttctccaactgctataagtacgcccctcctgaccatgag

SEQ ID NO: 13 - DNA, 21 bp, Artificial Sequence
  Synthetic Polynucleotide
cctggagatgacatagtctta

SEQ ID NO: 14 - DNA, 21 bp, Artificial Sequence
  Synthetic Polynucleotide
ccaaccaaagtcagttccttc

SEQ ID NO: 15 - DNA, 51 bp, Artificial Sequence
  Synthetic Polynucleotide
gccccgcccgcatccagcgacgccagcagcgatgcctccgcggacagtgac

SEQ ID NO: 16 - DNA, 51 bp, Artificial Sequence
  Synthetic Polynucleotide
gtcactgtccgcggaggcatcgctgctggcgtcgctggatgcgggcggggc

SEQ ID NO: 17 - DNA, 48 bp, Artificial Sequence
  Synthetic Polynucleotide
tccgcggacagtgacgctgcgactgatgacgctgaggaggagcgagcc

SEQ ID NO: 18 - DNA, 48 bp, Artificial Sequence
  Synthetic Polynucleotide
ggctcgctcctcctcagcgtcatcagtcgcagcgtcactgtccgcgga

SEQ ID NO: 19 - DNA, 51 bp, Artificial Sequence
  Synthetic Polynucleotide
gccccgcccgattccagcgacgacagcagcgatgactccgacgacagtgac

SEQ ID NO: 20 - DNA, 51 bp, Artificial Sequence
  Synthetic Polynucleotide
gtcactgtcgtcggagtcatcgctgctgtcgtcgctggaatcgggcggggc

SEQ ID NO: 21 - DNA, 48 bp, Artificial Sequence
  Synthetic Polynucleotide
tccgacgacagtgacgatgacactgatgacgatgaggaggagcgagcc

SEQ ID NO: 22 - DNA, 48 bp, Artificial Sequence
  Synthetic Polynucleotide
ggctcgctcctcctcatcgtcatcagtgtcatcgtcactgtcgtcgga

SEQ ID NO: 23 - DNA, 21 bp, Artificial Sequence
  Synthetic Polynucleotide
cccatgttgttctttgttatt